European Patent Application EP 4 151 651 A1, published March 22, 2023. Title: METHOD FOR IMPROVING AFFINITY OF ANTI-CYTOKINE ANTIBODY FOR ANTIGEN, METHOD FOR PRODUCING ANTI-CYTOKINE ANTIBODY, AND ANTI-CYTOKINE ANTIBODY. Applicant: SYSMEX CORPORATION. Application EP. The sequence listing filed with the application follows.

SEQUENCE LISTING (59 sequences)

SEQ ID NO: 1 - DNA, 20 bp, synthetic construct
  misc_feature 1..20: note = antisence oligo DNA
  source 1..20: mol_type = other DNA
gtaagctccctaatgtgctg

SEQ ID NO: 2 - DNA, 17 bp, synthetic construct
  misc_feature 1..17: note = primer
  source 1..17: mol_type = other DNA
ggttttcccagtcacga

SEQ ID NO: 3 - DNA, 20 bp, synthetic construct
  misc_feature 1..20: note = primer
  source 1..20: mol_type = other DNA
aggaaacagctatgaccatg

SEQ ID NO: 4 - protein, 225 aa, Mus musculus
EVQLQQSGPELVKPGASVKMSCKASGYTFTSYVMHWVKQKPGQGLEWIGYINPYNDGTKYNEKFKGKATLTSDKSSSTAYMELSSLTSEDSAVYYCAREGYGNLERDCWGQGTSVTVSSASTKGPSVFPLAPSSKSTSGGTAALGCLVKDYFPEPVTVSWNSGALTSGVHTFPAVLQSSGLYSLSSVVTVPSSSLGTQTYICNVNHKPSNTKVDKKVEPKSCDKT

SEQ ID NO: 5 - protein, 112 aa, Mus musculus
DIVLTQSPASLAVSLGQRATISCRASESVDGFGISFMNWFQQKPGQPPKLLIYVASNQGSGVPARFSGSGSGTDFSLNIHPMEEDDSAMYFCQQSKEVPWTFGGGTKLEIKR

SEQ ID NO: 6 - protein, 7 aa, Mus musculus
GYTFTSY

SEQ ID NO: 7 - protein, 4 aa, Mus musculus
PYND

SEQ ID NO: 8 - protein, 8 aa, Mus musculus
GYGNLERD

SEQ ID NO: 9 - protein, 11 aa, Mus musculus
SESVDGFGISF

SEQ ID NO: 10 - protein, 6 aa, Mus musculus
SKEVPW

SEQ ID NO: 11 - protein, 225 aa, Mus musculus
DVQLQESGPGLVKPSQTVSLTCTVTGISITTGNYRWSWIRQFPGNKLEWIGYIYYSGAITYNPSLTSRTTITRDTSMNQFFLEMISLTAEDTATYYCARDRYDYAVDFWGQGTSVTVSSASTKGPSVFPLAPSSKSTSGGTAALGCLVKDYFPEPVTVSWNSGALTSGVHTFPAVLQSSGLYSLSSVVTVPSSSLGTQTYICNVNHKPSNTKVDKKVEPKSCDKT

SEQ ID NO: 12 - protein, 108 aa, Mus musculus
DIQMTQSPASLSASVGETVTITCRSSENIYSFLTWFQQRQGKSPHLLVYYANTLAEGVPSRFSGSGSGTQFSLQINSLQPEDFGTYYCQHHYGTPWTFGGGTRLEIKR

SEQ ID NO: 13 - protein, 9 aa, Mus musculus
GISITTGNY

SEQ ID NO: 14 - protein, 7 aa, Mus musculus
RYDYAVD

SEQ ID NO: 15 - protein, 6 aa, Mus musculus
SENISF

SEQ ID NO: 16 - protein, 6 aa, Mus musculus
HYGTPW

SEQ ID NO: 17 - protein, 226 aa, Mus musculus
EVKLVESGGGLVKPGGSLKLSCAASGFTFNNYAMSWVRQTPEKRLEWVASISSGGNTYYPDSVKGRFTLSRDNARNILYLQMSRLRSEDTAMYYCARDKLRLPNWYFDVWGAGTTVTVSSASTKGPSVFPLAPSSKSTSGGTAALGCLVKDYFPEPVTVSWNSGALTSGVHTFPAVLQSSGLYSLSSVVTVPSSSLGTQTYICNVNHKPSNTKVDKKVEPKSCDKT

SEQ ID NO: 18 - protein, 112 aa, Mus musculus
DIVLTQSPPSLAVSLGQRATISCKASQSVDYDGDSYMNWYQQKPGQPPKVLIYGASNLESGIPARFSGSGSGTDFTLNIYPVEEEDAATYYCQQSNEDPPTFGGGTKLEIKR

SEQ ID NO: 19 - protein, 7 aa, Mus musculus
GFTFNNY

SEQ ID NO: 20 - protein, 13 aa, Mus musculus
SGGKLRLPNWYFD

SEQ ID NO: 21 - protein, 11 aa, Mus musculus
SQSVDYDGDSY

SEQ ID NO: 22 - protein, 6 aa, Mus musculus
SNEDPP

SEQ ID NO: 23 - protein, 225 aa, Mus musculus
EVQLVESGGGLVKPGGSLKLSCAASGFTFSSYAMSWVRQTPEKRLEWVATISNGGSYTYYPDSLKGRFTISRDNAKNTLYLQMSSLRSEDTAIYYCARGITGGVYFDYWGQGTTLTVSSASTKGPSVFPLAPSSKSTSGGTAALGCLVKDYFPEPVTVSWNSGALTSGVHTFPAVLQSSGLYSLSSVVTVPSSSLGTQTYICNVNHKPSNTKVDKKVEPKSCDKT

SEQ ID NO: 24 - protein, 108 aa, Mus musculus
DIQMTQSPASLSASVGETVTITCRASENIYSYLAWYQQKQGKSPHLLVYDAETLAEGVPSRFSGSGSGTQFSLKINSLQPEDFGSYYCQHHYGTPWTFGGGTKLEIKR

SEQ ID NO: 25 - protein, 7 aa, Mus musculus
GFTFSSY

SEQ ID NO: 26 - protein, 4 aa, Mus musculus
NGGS

SEQ ID NO: 27 - protein, 8 aa, Mus musculus
ITGGVYFD

SEQ ID NO: 28 - protein, 7 aa, Mus musculus
SENIYSY

SEQ ID NO: 29 - protein, 6 aa, Mus musculus
HYGTPW

SEQ ID NO: 30 - protein, 227 aa, Mus musculus
EVQLQESGPSLVKPSQTLSLTCSVTGDSITSGYWNWIRKFPGNKLEYMGYISYSGSTYYNPSLKSRISITRDTSKNQNYLQLNSVTTEDTATYYCARRDTTVVVPYYFDYWGQGTTLTVSSASTKGPSVFPLAPSSKSTSGGTAALGCLVKDYFPEPVTVSWNSGALTSGVHTFPAVLQSSGLYSLSSVVTVPSSSLGTQTYICNVNHKPSNTKVDKKVEPKSCDKT

SEQ ID NO: 31 - protein, 108 aa, Mus musculus
DIVMTQSHKFMSTSVGDRVSITCKASQDVGTAVAWYQQKPGQSPKLLIYWASTRHTGVPGRFTGSGSGTDFTLTINNVQSEDLADYFCQQYSSYPLTFGAGTKLELKR

SEQ ID NO: 32 - protein, 7 aa, Mus musculus
GDSITSG

SEQ ID NO: 33 - protein, 11 aa, Mus musculus
DTTVVVPYYFD

SEQ ID NO: 34 - protein, 7 aa, Mus musculus
SQDVGTA

SEQ ID NO: 35 - protein, 6 aa, Mus musculus
YSSYPL

SEQ ID NO: 36 - protein, 453 aa, Homo sapiens
AVQLQQSGPELVKPGASVKISCKASGYSFTSYWIHWIKQRPGQGLEWIGMIDPSDGETRLNQRFQGRATLTVDESTSTAYMQLRSPTSEDSAVYYCTRLKEYGNYDSFYFDVWGAGTLVTVSSASTKGPSVFPLAPSSKSTSGGTAALGCLVKDYFPEPVTVSWNSGALTSGVHTFPAVLQSSGLYSLSSVVTVPSSSLGTQTYICNVNHKPSNTKVDKKVEPKSCDKTHTCPPCPAPELLGGPSVFLFPPKPKDTLMISRTPEVTCVVVDVSHEDPEVKFNWYVDGVEVHNAKTKPREEQYNSTYRVVSVLTVLHQDWLNGKEYKCKVSNKALPAPIEKTISKAKGQPREPQVYTLPPSRDELTKNQVSLTCLVKGFYPSDIAVEWESNGQPENNYKTTPPVLDSDGSFFLYSKLTVDKSRWQQGNVFSCSVMHEALHNHYTQKSLSLSPGK

SEQ ID NO: 37 - protein, 214 aa, Homo sapiens
DIQMTQSPASLSVSVGDTITLTCHASQNIDVWLSWFQQKPGNIPKLLIYKASNLHTGVPSRFSGSGSGTGFTLTISSLQPEDIATYYCQQAHSYPFTFGGGTKLEIKRTVAAPSVFIFPPSDEQLKSGTASVVCLLNNFYPREAKVQWKVDNALQSGNSQESVTEQDSKDSTYSLSSTLTLSKADYEKHKVYACEVTHQGLSSPVTMSFNRGEC

SEQ ID NO: 38 - protein, 7 aa, Homo sapiens
GYSFTSY

SEQ ID NO: 39 - protein, 4 aa, Homo sapiens
PSDG

SEQ ID NO: 40 - protein, 12 aa, Homo sapiens
KEYGNYDSFYFD

SEQ ID NO: 41 - protein, 7 aa, Homo sapiens
SQNIDVW

SEQ ID NO: 42 - protein, 6 aa, Homo sapiens
AHSYPF

SEQ ID NO: 43 - protein, 112 aa, synthetic construct
  REGION 1..112: note = modified antibody
DIVLTQSPASLAVSLGQRATISCRASESVDGFGISFMNWFQQKPGQPPKLLIYVASNQGSGVPARFRGRGRGTDFSLNIHPMEEDDSAMYFCQQSKEVPWTFGGGTKLEIKR

SEQ ID NO: 44 - protein, 112 aa, synthetic construct
  REGION 1..112: note = modified antibody
DIVLTQSPASLAVSLGQRATISCRASESVDGFGISFMNWFQQKPGQPPKLLIYVASNQGSGVPARFRGRGRGTRFSLNIHPMEEDDSAMYFCQQSKEVPWTFGGGTKLEIKR

SEQ ID NO: 45 - protein, 112 aa, synthetic construct
  REGION 1..112: note = modified antibody
DIVLTQSPASLAVSLGQRATISCRASESVDGFGISFMNWFQQKPGQPPKLLIYVASNQGSGVPARFRGRGRGTRFRLNIHPMEEDDSAMYFCQQSKEVPWTFGGGTKLEIKR

SEQ ID NO: 46 - protein, 108 aa, synthetic construct
  REGION 1..108: note = modified antibody
DIQMTQSPASLSASVGETVTITCRSSENIYSFLTWFQQRQGKSPHLLVYYANTLAEGVPSRFRGRGRGTQFSLQINSLQPEDFGTYYCQHHYGTPWTFGGGTRLEIKR

SEQ ID NO: 47 - protein, 108 aa, synthetic construct
  REGION 1..108: note = modified antibody
DIQMTQSPASLSASVGETVTITCRSSENIYSFLTWFQQRQGKSPHLLVYYANTLAEGVPSRFRGRGRGTRFSLQINSLQPEDFGTYYCQHHYGTPWTFGGGTRLEIKR

SEQ ID NO: 48 - protein, 108 aa, synthetic construct
  REGION 1..108: note = modified antibody
DIQMTQSPASLSASVGETVTITCRSSENIYSFLTWFQQRQGKSPHLLVYYANTLAEGVPSRFRGRGRGTRFRLQINSLQPEDFGTYYCQHHYGTPWTFGGGTRLEIKR

SEQ ID NO: 49 - protein, 112 aa, synthetic construct
  REGION 1..112: note = modified antibody
DIVLTQSPPSLAVSLGQRATISCKASQSVDYDGDSYMNWYQQKPGQPPKVLIYGASNLESGIPARFRGRGRGTDFTLNIYPVEEEDAATYYCQQSNEDPPTFGGGTKLEIKR

SEQ ID NO: 50 - protein, 112 aa, synthetic construct
  REGION 1..112: note = modified antibody
DIVLTQSPPSLAVSLGQRATISCKASQSVDYDGDSYMNWYQQKPGQPPKVLIYGASNLESGIPARFRGRGRGTRFTLNIYPVEEEDAATYYCQQSNEDPPTFGGGTKLEIKR

SEQ ID NO: 51 - protein, 112 aa, synthetic construct
  REGION 1..112: note = modified antibody
DIVLTQSPPSLAVSLGQRATISCKASQSVDYDGDSYMNWYQQKPGQPPKVLIYGASNLESGIPARFRGRGRGTRFRLNIYPVEEEDAATYYCQQSNEDPPTFGGGTKLEIKR

SEQ ID NO: 52 - protein, 108 aa, synthetic construct
  REGION 1..108: note = modified antibody
DIQMTQSPASLSASVGETVTITCRASENIYSYLAWYQQKQGKSPHLLVYDAETLAEGVPSRFRGRGRGTQFSLKINSLQPEDFGSYYCQHHYGTPWTFGGGTKLEIKR

SEQ ID NO: 53 - protein, 108 aa, synthetic construct
  REGION 1..108: note = modified antibody
DIQMTQSPASLSASVGETVTITCRASENIYSYLAWYQQKQGKSPHLLVYDAETLAEGVPSRFRGRGRGTRFSLKINSLQPEDFGSYYCQHHYGTPWTFGGGTKLEIKR

SEQ ID NO: 54 - protein, 108 aa, synthetic construct
  REGION 1..108: note = modified antibody
DIQMTQSPASLSASVGETVTITCRASENIYSYLAWYQQKQGKSPHLLVYDAETLAEGVPSRFRGRGRGTRFRLKINSLQPEDFGSYYCQHHYGTPWTFGGGTKLEIKR

SEQ ID NO: 55 - protein, 108 aa, synthetic construct
  REGION 1..108: note = modified antibody
DIVMTQSHKFMSTSVGDRVSITCKASQDVGTAVAWYQQKPGQSPKLLIYWASTRHTGVPGRFRGRGRGTDFTLTINNVQSEDLADYFCQQYSSYPLTFGAGTKLELKR

SEQ ID NO: 56 - protein, 108 aa, synthetic construct
  REGION 1..108: note = modified antibody
DIVMTQSHKFMSTSVGDRVSITCKASQDVGTAVAWYQQKPGQSPKLLIYWASTRHTGVPGRFRGRGRGTRFTLTINNVQSEDLADYFCQQYSSYPLTFGAGTKLELKR

SEQ ID NO: 57 - protein, 108 aa, synthetic construct
  REGION 1..108: note = modified antibody
DIVMTQSHKFMSTSVGDRVSITCKASQDVGTAVAWYQQKPGQSPKLLIYWASTRHTGVPGRFRGRGRGTRFRLTINNVQSEDLADYFCQQYSSYPLTFGAGTKLELKR

SEQ ID NO: 58 - protein, 214 aa, synthetic construct
  REGION 1..214: note = modified antibody
DIQMTQSPASLSVSVGDTITLTCHASQNIDVWLSWFQQKPGNIPKLLIYKASNLHTGVPSRFRGRGRGTGFTLTISSLQPEDIATYYCQQAHSYPFTFGGGTKLEIKRTVAAPSVFIFPPSDEQLKSGTASVVCLLNNFYPREAKVQWKVDNALQSGNSQESVTEQDSKDSTYSLSSTLTLSKADYEKHKVYACEVTHQGLSSPVTMSFNRGEC

SEQ ID NO: 59 - protein, 214 aa, synthetic construct
  REGION 1..214: note = modified antibody
DIQMTQSPASLSVSVGDTITLTCHASQNIDVWLSWFQQKPGNIPKLLIYKASNLHTGVPSRFRGRGRGTRFTLTISSLQPEDIATYYCQQAHSYPFTFGGGTKLEIKRTVAAPSVFIFPPSDEQLKSGTASVVCLLNNFYPREAKVQWKVDNALQSGNSQESVTEQDSKDSTYSLSSTLTLSKADYEKHKVYACEVTHQGLSSPVTMSFNRGEC